European Patent Application EP 4 438 125 A2, published October 2, 2024. Title: CONJUGATE OF GALNAC AND SAPONIN, THERAPEUTIC COMPOSITION COMPRISING SAID CONJUGATE AND A GALNAC-OLIGONUCLEOTIDE CONJUGATE. Applicant: Sapreme Technologies B.V. Application EP, filed June 18, 2021. The sequence listing filed with the application follows.

SEQUENCE LISTING (20 sequences)

SEQ ID NO: 1 - DNA, 16 bp, synthetic construct
  source 1..16: mol_type = other DNA; note = Antisense BNA (HSP27) oligo nucleic acid sequence
ggcacagccagtggcg

SEQ ID NO: 2 - DNA, 20 bp, synthetic construct
  source 1..20: mol_type = other DNA; note = APOB BNA oligo
gcctcagtctgcttcgcacc

SEQ ID NO: 3 - DNA, 20 bp, synthetic construct
  source 1..20: mol_type = other DNA; note = APOB scrambled BNA oligo
ggcctctctacaccgctcgt

SEQ ID NO: 4 - DNA, 20 bp, synthetic construct
  source 1..20: mol_type = other DNA; note = HSP27 primer forward sequence
gcagtccaacgagatcacca

SEQ ID NO: 5 - DNA, 20 bp, synthetic construct
  source 1..20: mol_type = other DNA; note = HSP27 primer reverse sequence
taaggctttacttggcggca

SEQ ID NO: 6 - DNA, 20 bp, synthetic construct
  source 1..20: mol_type = other DNA; note = ApoB primer forward sequence
agggtccgggaatctgatga

SEQ ID NO: 7 - DNA, 21 bp, synthetic construct
  source 1..21: mol_type = other DNA; note = ApoB primer reverse sequence
tgggcacgttgtctttcagag

SEQ ID NO: 8 - DNA, 20 bp, synthetic construct
  source 1..20: mol_type = other DNA; note = HBMS primer forward sequence
cacccacacacagcctactt

SEQ ID NO: 9 - DNA, 20 bp, synthetic construct
  source 1..20: mol_type = other DNA; note = HBMS primer reverse sequence
gtacccacgcgaatcactct

SEQ ID NO: 10 - DNA, 22 bp, synthetic construct
  source 1..22: mol_type = other DNA; note = GUSB primer forward sequence
gaaaatacgtggttggagagct

SEQ ID NO: 11 - DNA, 22 bp, synthetic construct
  source 1..22: mol_type = other DNA; note = GUSB primer reverse sequence
ccgagtgaagatccccttttta

SEQ ID NO: 12 - DNA, 13 bp, synthetic construct
  source 1..13: mol_type = other DNA; note = ApoB#02
gcattggtattca

SEQ ID NO: 13 - DNA, 24 bp, synthetic construct
  source 1..24: mol_type = other DNA; note = ApoB#02 forward primer
gctaacactaagaaccagaagatc

SEQ ID NO: 14 - DNA, 20 bp, synthetic construct
  source 1..20: mol_type = other DNA; note = ApoB#02 reverse primer
tgtccgtctaaggatcctgc

SEQ ID NO: 15 - DNA, 18 bp, synthetic construct
  source 1..18: mol_type = other DNA; note = Mm PPIA forward primer
gcggcaggtccatctacg

SEQ ID NO: 16 - DNA, 19 bp, synthetic construct
  source 1..19: mol_type = other DNA; note = Mm PPIA reverse primer
gccatccagccattcagtc

SEQ ID NO: 17 - DNA, 20 bp, synthetic construct
  source 1..20: mol_type = other DNA; note = Mm SDHA forward primer
gaggaagcacaccctctcat

SEQ ID NO: 18 - DNA, 20 bp, synthetic construct
  source 1..20: mol_type = other DNA; note = Mm SDHA reverse primer
ggagcggatagcaggaggta

SEQ ID NO: 19 - DNA, 20 bp, synthetic construct
  source 1..20: mol_type = other DNA; note = Mm RSP17 forward primer
gtgcgaggagatcgccatta

SEQ ID NO: 20 - DNA, 20 bp, synthetic construct
  source 1..20: mol_type = other DNA; note = Mm RSP17 reverse primer
atccgcttcatcagatgcgt